European Patent Specification EP 4 010 356 B1, published September 4, 2024. Title: METHODS AND COMPOSITIONS FOR DUAL GLYCAN BINDING AAV2.5 VECTOR. Applicant: THE UNIVERSITY OF NORTH CAROLINA AT CHAPEL HILL Samulski, Richard J. The sequence listing filed with the application follows.

SEQUENCE LISTING (2 sequences)

SEQ ID NO: 1 - protein, 736 aa, Artificial Sequence
  AAV2.5 capsid protein
MAADGYLPDWLEDTLSEGIRQWWKLKPGPPPPKPAERHKDDSRGLVLPGYKYLGPFNGLDKGEPVNEADAAALEHDKAYDRQLDSGDNPYLKYNHADAEFQERLKEDTSFGGNLGRAVFQAKKRVLEPLGLVEEPVKTAPGKKRPVEHSPVEPDSSSGTGKAGQQPARKRLNFGQTGDADSVPDPQPLGQPPAAPSGLGTNTMATGSGAPMADNNEGADGVGNSSGNWHCDSTWMGDRVITTSTRTWALPTYNNHLYKQISSASTGASNDNHYFGYSTPWGYFDFNRFHCHFSPRDWQRLINNNWGFRPKRLNFKLFNIQVKEVTQNDGTTTIANNLTSTVQVFTDSEYQLPYVLGSAHQGCLPPFPADVFMVPQYGYLTLNNGSQAVGRSSFYCLEYFPSQMLRTGNNFTFSYTFEDVPFHSSYAHSQSLDRLMNPLIDQYLYYLSRTNTPSGTTTQSRLQFSQAGASDIRDQSRNWLPGPCYRQQRVSKTSADNNNSEYSWTGATKYHLNGRDSLVNPGPAMASHKDDEEKFFPQSGVLIFGKQGSEKTNVDIEKVMITDEEEIRTTNPVATEQYGSVSTNLQRGNRQAATADVNTQGVLPGMVWQDRDVYLQGPIWAKIPHTDGHFHPSPLMGGFGLKHPPPQILIKNTPVPANPSTTFSAAKFASFITQYSTGQVSVEIEWELQKENSKRWNPEIQYTSNYAKSANVDFTVDNNGVYSEPRPIGTRYLTRNL

SEQ ID NO: 2 - protein, 736 aa, Artificial Sequence
  AAV2.5G9 A267 capsid protein
MAADGYLPDWLEDTLSEGIRQWWKLKPGPPPPKPAERHKDDSRGLVLPGYKYLGPFNGLDKGEPVNEADAAALEHDKAYDRQLDSGDNPYLKYNHADAEFQERLKEDTSFGGNLGRAVFQAKKRVLEPLGLVEEPVKTAPGKKRPVEHSPVEPDSSSGTGKAGQQPARKRLNFGQTGDADSVPDPQPLGQPPAAPSGLGTNTMATGSGAPMADNNEGADGVGNSSGNWHCDSTWMGDRVITTSTRTWALPTYNNHLYKQISSASTGASNDNHYFGYSTPWGYFDFNRFHCHFSPRDWQRLINNNWGFRPKRLNFKLFNIQVKEVTQNDGTTTIANNLTSTVQVFTDSEYQLPYVLGSAHQGCLPPFPADVFMVPQYGYLTLNNGSQAVGRSSFYCLEYFPSQMLRTGNNFTFSYTFEDVPFHSSYAHSQSLDRLMNPLIDQYLYYLSRTNTPSGTTTQSRLQFSVAGPSNMAVQGRNWLPGPCYRQQRVSKTSADNNNSEFAWTGATKYHLNGRDSLVNPGPAMASHKDDEEKFFPQSGVLIFGKQGSEKTNVDIEKVMITDEEEIRTTNPVATEQYGSVSTNLQRGNRQAATADVNTQGVLPGMVWQDRDVYLQGPIWAKIPHTDGHFHPSPLMGGFGLKHPPPQILIKNTPVPANPSTTFSAAKFASFITQYSTGQVSVEIEWELQKENSKRWNPEIQYTSNYAKSANVDFTVDNNGVYSEPRPIGTRYLTRNL